European Patent Application EP 4 647 081 A1, published November 12, 2025. Title: CELL SURFACE IG-AIMED IMMUNE MEMORY ERASERS AND USES THEREOF. Applicant: IFOM - Istituto Fondazione di Oncologia Molecolare ETS. The sequence listing filed with the application follows.

SEQUENCE LISTING (26 sequences)

SEQ ID NO: 1 - protein, 533 aa, synthetic construct
MGADDVVDSSKSFVMENFSSYHGTKPGYVDSIQKGIQKPKSGTQGNYDDDWKGFYSTDNKYDAAGYSVDNENPLSGKAGGVVKVTYPGLTKVLALKVDNAETIKKELGLSLTEPLMEQVGTEEFIKRFGDGASRVVLSLPFAEGSSSVEYINNWEQAKALSVELEINFETRGKRGQDAMYEYMAQACAGNRVRRSVGSSLSCINLDWDVIRDKTKTKIESLKEHGPIKNKMSESPNKTVSEEKAKQYLEEFHQTALEHPELSELKTVTGTNPVFAGANYAAWAVNVAQVIDSETADNLEKTTAALSILPGIGSVMGIADGAVHHNTEEIVAQSIALSSLMVAQAIPLVGELVDIGFAAYNFVESIINLFQVVHNSYNRPAYSPGHKTSSGGGSSGGGSAVDNKFNKEQQNAFYEILHLPNLNEEQRNAFIQSLKDDPSQSANLLAEAKKLNDAQAPKVDNKFNKEQQNAFYEILHLPNLNEEQRNAFIQSLKDDPSQSANLLAEAKKLNGAQAPKVDANSAGKSTLEHHHHHH

SEQ ID NO: 2 - protein, 533 aa, synthetic construct
MGADDVVDSSKSFVMENFSSYHGTKPGYVDSIQKGIQKPKSGTQGNYDDDWKGFYSTDNKYDAAGYSVDNENPLSGKAGGVVKVTYPGLTKVLALKVDNAETIKKELGLSLTEPLMEQVGTEEFIKRFGDGASRVVLSLPFAEGSSSVEYINNWEQAKALSVELEINFETRGKRGQDAMYEYMAQACAGNRVRRSVGSSLSCINLDWDVIRDKTKTKIESLKEHGPIKNKMSESPNKTVSEEKAKQYLEEFHQTALEHPELSELKTVTGTNPVFAGANYAAWAVNVAQVIDSETADNLEKTTAALSILPGIGSVMGIADGAVHHNTEEIVAQSIALSSLMVAQAIPLVGELVDIGFAAYNFVESIINLFQVVHNSYNRPAYSPGHKTSSGGGSSGGGSAVDNKFNKETIQASQEIRLLPNLNGRQKLAFIHSLLDDPSQSANLLAEAKKLNDAQAPKVDNKFNKETIQASQEIRLLPNLNGRQKLAFIHSLLDDPSQSANLLAEAKKLNGAQAPKVDANSAGKSTLEHHHHHH

SEQ ID NO: 3 - protein, 489 aa, synthetic construct
MGADDVVDSSKSFVMENFSSYHGTKPGYVDSIQKGIQKPKSGTQGNYDDDWKGFYSTDNKYDAAGYSVDNENPLSGKAGGVVKVTYPGLTKVLALKVDNAETIKKELGLSLTEPLMEQVGTEEFIKRFGDGASRVVLSLPFAEGSSSVEYINNWEQAKALSVELEINFETRGKRGQDAMYEYMAQACAGNRVRRSVGSSLSCINLDWDVIRDKTKTKIESLKEHGPIKNKMSESPNKTVSEEKAKQYLEEFHQTALEHPELSELKTVTGTNPVFAGANYAAWAVNVAQVIDSETADNLEKTTAALSILPGIGSVMGIADGAVHHNTEEIVAQSIALSSLMVAQAIPLVGELVDIGFAAYNFVESIINLFQVVHNSYNRPAYSPGHKTSSGGGSSGGGSAASMADDMERIFKRFDTNGDGKISLSELTDALRTLGSTSADEVQRMMAEIDTDGDGFIDFNEFISFCNANPGLMKDVAKVFVDLEHHHHHH

SEQ ID NO: 4 - protein, 387 aa, synthetic construct
MGADDVVDSSKSFVMENFSSYHGTKPGYVDSIQKGIQKPKSGTQGNYDDDWKGFYSTDNKYDAAGYSVDNENPLSGKAGGVVKVTYPGLTKVLALKVDNAETIKKELGLSLTEPLMEQVGTEEFIKRFGDGASRVVLSLPFAEGSSSVEYINNWEQAKALSVELEINFETRGKRGQDAMYEYMAQACAGNRVRRSVGSSLSCINLDWDVIRDKTKTKIESLKEHGPIKNKMSESPNKTVSEEKAKQYLEEFHQTALEHPELSELKTVTGTNPVFAGANYAAWAVNVAQVIDSETADNLEKTTAALSILPGIGSVMGIADGAVHHNTEEIVAQSIALSSLMVAQAIPLVGELVDIGFAAYNFVESIINLFQVVHNSYNRPAYSPGHKT

SEQ ID NO: 5 - protein, 12 aa, synthetic construct
SSGGGSSGGGSA

SEQ ID NO: 6 - protein, 116 aa, synthetic construct
VDNKFNKEQQNAFYEILHLPNLNEEQRNAFIQSLKDDPSQSANLLAEAKKLNDAQAPKVDNKFNKEQQNAFYEILHLPNLNEEQRNAFIQSLKDDPSQSANLLAEAKKLNGAQAPK

SEQ ID NO: 7 - protein, 6 aa, synthetic construct
HHHHHH

SEQ ID NO: 8 - DNA, 1602 bp, synthetic construct
  source 1..1602: mol_type = other DNA
atgggcgctgatgatgttgttgattcttctaaatcttttgtgatggaaaacttttcttcgtaccacgggactaaacctggttatgtagattccattcaaaaaggtatacaaaagccaaaatctggtacacaaggaaattatgacgatgattggaaagggttttatagtaccgacaataaatacgacgctgcgggatactctgtagataatgaaaacccgctctctggaaaagctggaggcgtggtcaaagtgacgtatccaggactgacgaaggttctcgcactaaaagtggataatgccgaaactattaagaaagagttaggtttaagtctcactgaaccgttgatggagcaagtcggaacggaagagtttatcaaaaggttcggtgatggtgcttcgcgtgtagtgctcagccttcccttcgctgaggggagttctagcgttgaatatattaataactgggaacaggcgaaagcgttaagcgtagaacttgagattaattttgaaacccgtggaaaacgtggccaagatgcgatgtatgagtatatggctcaagcctgtgcaggaaatcgtgtcaggcgatcagtaggtagctcattgtcatgcataaatcttgattgggatgtcataagggataaaactaagacaaagatagagtctttgaaagagcatggccctatcaaaaataaaatgagcgaaagtcccaataaaacagtatctgaggaaaaagctaaacaatacctagaagaatttcatcaaacggcattagagcatcctgaattgtcagaacttaaaaccgttactgggaccaatcctgtattcgctggggctaactatgcggcgtgggcagtaaacgttgcgcaagttatcgatagcgaaacagctgataatttggaaaagacaactgctgctctttcgatacttcctggtatcggtagcgtaatgggcattgcagacggtgccgttcaccacaatacagaagagatagtggcacaatcaatagctttatcgtctttaatggttgctcaagctattccattggtaggagagctagttgatattggtttcgctgcatataattttgtagagagtattatcaatttatttcaagtagttcataattcgtataatcgtcccgcgtattctccggggcataaaacgtctagcggaggtggctctagcggtggaggatccgcagtggacaacaaattcaacaaagaacaacaaaacgcgttctatgagatcttacatttacctaacttaaacgaagaacaacgaaacgccttcatccaaagtttaaaagatgacccaagccaaagcgctaaccttttagcagaagctaaaaagctaaatgatgctcaggcgccgaaagtagacaacaaattcaacaaagaacaacaaaacgcgttctatgagatcttacatttacctaacttaaacgaagaacaacgaaacgccttcatccaaagtttaaaagatgacccaagccaaagcgctaaccttttagcagaagctaaaaagctaaatggtgctcaggcgccgaaagtagacgcgaattccgcggggaagtcaaccctcgagcaccaccaccaccaccactga

SEQ ID NO: 9 - DNA, 1161 bp, synthetic construct
  source 1..1161: mol_type = other DNA
atgggcgctgatgatgttgttgattcttctaaatcttttgtgatggaaaacttttcttcgtaccacgggactaaacctggttatgtagattccattcaaaaaggtatacaaaagccaaaatctggtacacaaggaaattatgacgatgattggaaagggttttatagtaccgacaataaatacgacgctgcgggatactctgtagataatgaaaacccgctctctggaaaagctggaggcgtggtcaaagtgacgtatccaggactgacgaaggttctcgcactaaaagtggataatgccgaaactattaagaaagagttaggtttaagtctcactgaaccgttgatggagcaagtcggaacggaagagtttatcaaaaggttcggtgatggtgcttcgcgtgtagtgctcagccttcccttcgctgaggggagttctagcgttgaatatattaataactgggaacaggcgaaagcgttaagcgtagaacttgagattaattttgaaacccgtggaaaacgtggccaagatgcgatgtatgagtatatggctcaagcctgtgcaggaaatcgtgtcaggcgatcagtaggtagctcattgtcatgcataaatcttgattgggatgtcataagggataaaactaagacaaagatagagtctttgaaagagcatggccctatcaaaaataaaatgagcgaaagtcccaataaaacagtatctgaggaaaaagctaaacaatacctagaagaatttcatcaaacggcattagagcatcctgaattgtcagaacttaaaaccgttactgggaccaatcctgtattcgctggggctaactatgcggcgtgggcagtaaacgttgcgcaagttatcgatagcgaaacagctgataatttggaaaagacaactgctgctctttcgatacttcctggtatcggtagcgtaatgggcattgcagacggtgccgttcaccacaatacagaagagatagtggcacaatcaatagctttatcgtctttaatggttgctcaagctattccattggtaggagagctagttgatattggtttcgctgcatataattttgtagagagtattatcaatttatttcaagtagttcataattcgtataatcgtcccgcgtattctccggggcataaaacg

SEQ ID NO: 10 - DNA, 36 bp, synthetic construct
  source 1..36: mol_type = other DNA
tctagcggaggtggctctagcggtggaggatccgca

SEQ ID NO: 11 - DNA, 348 bp, synthetic construct
  source 1..348: mol_type = other DNA
gtggacaacaaattcaacaaagaacaacaaaacgcgttctatgagatcttacatttacctaacttaaacgaagaacaacgaaacgccttcatccaaagtttaaaagatgacccaagccaaagcgctaaccttttagcagaagctaaaaagctaaatgatgctcaggcgccgaaagtagacaacaaattcaacaaagaacaacaaaacgcgttctatgagatcttacatttacctaacttaaacgaagaacaacgaaacgccttcatccaaagtttaaaagatgacccaagccaaagcgctaaccttttagcagaagctaaaaagctaaatggtgctcaggcgccgaaa

SEQ ID NO: 12 - DNA, 18 bp, synthetic construct
  source 1..18: mol_type = other DNA
caccaccaccaccaccac

SEQ ID NO: 13 - protein, 115 aa, synthetic construct
VDNKFNKETIQASQEIRLLPNLNGRQKLAFIHSLLDDPSQSANLLAEAKKLNDAQAPKVDNKFNKETIQASQEIRLLPNLNGRQKLAFIHSLLDDPSQSANLLAEAKKLNGAQAP

SEQ ID NO: 14 - DNA, 1602 bp, synthetic construct
  source 1..1602: mol_type = other DNA
atgggcgctgatgatgttgttgattcttctaaatcttttgtgatggaaaacttttcttcgtaccacgggactaaacctggttatgtagattccattcaaaaaggtatacaaaagccaaaatctggtacacaaggaaattatgacgatgattggaaagggttttatagtaccgacaataaatacgacgctgcgggatactctgtagataatgaaaacccgctctctggaaaagctggaggcgtggtcaaagtgacgtatccaggactgacgaaggttctcgcactaaaagtggataatgccgaaactattaagaaagagttaggtttaagtctcactgaaccgttgatggagcaagtcggaacggaagagtttatcaaaaggttcggtgatggtgcttcgcgtgtagtgctcagccttcccttcgctgaggggagttctagcgttgaatatattaataactgggaacaggcgaaagcgttaagcgtagaacttgagattaattttgaaacccgtggaaaacgtggccaagatgcgatgtatgagtatatggctcaagcctgtgcaggaaatcgtgtcaggcgatcagtaggtagctcattgtcatgcataaatcttgattgggatgtcataagggataaaactaagacaaagatagagtctttgaaagagcatggccctatcaaaaataaaatgagcgaaagtcccaataaaacagtatctgaggaaaaagctaaacaatacctagaagaatttcatcaaacggcattagagcatcctgaattgtcagaacttaaaaccgttactgggaccaatcctgtattcgctggggctaactatgcggcgtgggcagtaaacgttgcgcaagttatcgatagcgaaacagctgataatttggaaaagacaactgctgctctttcgatacttcctggtatcggtagcgtaatgggcattgcagacggtgccgttcaccacaatacagaagagatagtggcacaatcaatagctttatcgtctttaatggttgctcaagctattccattggtaggagagctagttgatattggtttcgctgcatataattttgtagagagtattatcaatttatttcaagtagttcataattcgtataatcgtcccgcgtattctccggggcataaaacgtctagcggaggtggctctagcggtggaggatccgcagtggacaacaaattcaacaaagaaaccatccaggcgtcccaggagatccgtctgttacctaacttaaacggtcgtcaaaaactggccttcatccacagtttactggatgacccaagccaaagcgctaaccttttagcagaagctaaaaagctaaatgatgctcaggcgccgaaagtcgacaacaaattcaacaaagaaacgattcaggcgtctcaggagatccgcctgttacctaacttaaacggtcgccaaaaactggccttcatccatagtttactggatgacccaagccaaagcgctaaccttttagcagaagctaaaaagctaaatggtgctcaggcgccgaaagtagacgcgaattccgcggggaagtcaaccctcgagcaccaccaccaccaccactga

SEQ ID NO: 15 - DNA, 348 bp, synthetic construct
  source 1..348: mol_type = other DNA
gtggacaacaaattcaacaaagaaaccatccaggcgtcccaggagatccgtctgttacctaacttaaacggtcgtcaaaaactggccttcatccacagtttactggatgacccaagccaaagcgctaaccttttagcagaagctaaaaagctaaatgatgctcaggcgccgaaagtcgacaacaaattcaacaaagaaacgattcaggcgtctcaggagatccgcctgttacctaacttaaacggtcgccaaaaactggccttcatccatagtttactggatgacccaagccaaagcgctaaccttttagcagaagctaaaaagctaaatggtgctcaggcgccgaaa

SEQ ID NO: 16 - protein, 78 aa, synthetic construct
MADDMERIFKRFDTNGDGKISLSELTDALRTLGSTSADEVQRMMAEIDTDGDGFIDFNEFISFCNANPGLMKDVAKVF

SEQ ID NO: 17 - DNA, 1470 bp, synthetic construct
  source 1..1470: mol_type = other DNA
atgggcgctgatgatgttgttgattcttctaaatcttttgtgatggaaaacttttcttcgtaccacgggactaaacctggttatgtagattccattcaaaaaggtatacaaaagccaaaatctggtacacaaggaaattatgacgatgattggaaagggttttatagtaccgacaataaatacgacgctgcgggatactctgtagataatgaaaacccgctctctggaaaagctggaggcgtggtcaaagtgacgtatccaggactgacgaaggttctcgcactaaaagtggataatgccgaaactattaagaaagagttaggtttaagtctcactgaaccgttgatggagcaagtcggaacggaagagtttatcaaaaggttcggtgatggtgcttcgcgtgtagtgctcagccttcccttcgctgaggggagttctagcgttgaatatattaataactgggaacaggcgaaagcgttaagcgtagaacttgagattaattttgaaacccgtggaaaacgtggccaagatgcgatgtatgagtatatggctcaagcctgtgcaggaaatcgtgtcaggcgatcagtaggtagctcattgtcatgcataaatcttgattgggatgtcataagggataaaactaagacaaagatagagtctttgaaagagcatggccctatcaaaaataaaatgagcgaaagtcccaataaaacagtatctgaggaaaaagctaaacaatacctagaagaatttcatcaaacggcattagagcatcctgaattgtcagaacttaaaaccgttactgggaccaatcctgtattcgctggggctaactatgcggcgtgggcagtaaacgttgcgcaagttatcgatagcgaaacagctgataatttggaaaagacaactgctgctctttcgatacttcctggtatcggtagcgtaatgggcattgcagacggtgccgttcaccacaatacagaagagatagtggcacaatcaatagctttatcgtctttaatggttgctcaagctattccattggtaggagagctagttgatattggtttcgctgcatataattttgtagagagtattatcaatttatttcaagtagttcataattcgtataatcgtcccgcgtattctccggggcataaaacgtctagcggaggtggctctagcggtggaggatcagcagctagcatggcggacgacatggagaggatcttcaagaggttcgacacgaacggtgacgggaagatctctctgtcggagctgacggacgcactgcggacgctgggctcgacgtcggcggacgaggtgcagcgcatgatggcggagatcgacaccgacggcgacggcttcatcgacttcaacgagttcatctccttctgcaacgccaaccctggactcatgaaggacgtcgccaaggtcttcgtcgacctcgagcaccaccaccaccaccactga

SEQ ID NO: 18 - DNA, 234 bp, synthetic construct
  source 1..234: mol_type = other DNA
atggcggacgacatggagaggatcttcaagaggttcgacacgaacggtgacgggaagatctctctgtcggagctgacggacgcactgcggacgctgggctcgacgtcggcggacgaggtgcagcgcatgatggcggagatcgacaccgacggcgacggcttcatcgacttcaacgagttcatctccttctgcaacgccaaccctggactcatgaaggacgtcgccaaggtcttc

SEQ ID NO: 19 - protein, 10 aa, synthetic construct
GGGGSGGGGS

SEQ ID NO: 20 - protein, 15 aa, synthetic construct
GGGGSGGGGSGGGGS

SEQ ID NO: 21 - protein, 20 aa, synthetic construct
GGGGSGGGGSGGGGSGGGGS

SEQ ID NO: 22 - protein, 25 aa, synthetic construct
GGGGSGGGGSGGGGSGGGGSGGGGS

SEQ ID NO: 23 - protein, 16 aa, synthetic construct
SGGGGSGGGGSGGGGS

SEQ ID NO: 24 - protein, 15 aa, synthetic construct
GGGGSGGGGSGGGAS

SEQ ID NO: 25 - protein, 28 aa, synthetic construct
RRKRGSGLINEGRGSLLTCGDVEENPGP

SEQ ID NO: 26 - protein, 8 aa, synthetic construct
DYKDDDDK